European Patent Specification EP 4 076 499 B1, published July 16, 2025. Title: USE OF GLIAL CELL LINE-DERIVED NEUROTROPHIC FACTOR (GDNF) FOR THE TREATMENT OF ENTERIC NEUROPATHIES. Applicant: TRANSFERT PLUS, SOCIÉTÉ EN COMMANDITE. The sequence listing filed with the application follows.

SEQUENCE LISTING (3 sequences)

SEQ ID NO: 1 - protein, 211 aa, Homo sapiens
  SIGNAL (1)..(19)
  PROPEP (20)..(75)
MKLWDVVAVCLVLLHTASAFPLPAGKRPPEAPAEDRSLGRRRAPFALSSDSNMPEDYPDQFDDVMDFIQATIKRLKRSPDKQMAVLPRRERNRQAAAANPENSRGKGRRGQRGKNRGCVLTAIHLNVTDLGLGYETKEELIFRYCSGSCDAAETTYDKILKNLSRNRRLVSDKVGQACCRPIAFDDDLSFLDDNLVYHILRKHSAKRCGCI

SEQ ID NO: 2 - DNA, 4171 bp, Homo sapiens
agcctgcgctcctggcgccctcatgtcttcacgggactccccgcgccggttgacgtggtgtctcgttcggatctccaggcaagacctcagctccggcagcagcatcagacaaaccagtctcgtgctcccaggcagtgcgcccagaggaggcgcagagcgcggcagctgccgctgagccgcccgcagcgccccgggcccgcgcagccccagccaagagcgcgacgcgcgcagccctgtcagccccccacccaaagcagcggcggctgctcggacctcggcttctgggggtgcgggggcccggcgggagagttgccggcagccctcgccctgttggcggcggcggcggcgggagtcttggccgccgcctccagcgcgcccttgctgccccgcgcgaccccaggattgcgaactcttgcccctgacctgttgggcggggctccgcgctccagccatcagcccggatgggtctcctggctgggacttggggcacctggagttaatgtccaacctagggtctgcggagacccgatccgaggtgccgccgccggacgggactttaagatgaagttatgggatgtcgtggctgtctgcctggtgctgctccacaccgcgtccgccttcccgctgcccgccggtaagaggcctcccgaggcgcccgccgaagaccgctccctcggccgccgccgcgcgcccttcgcgctgagcagtgactcaaatatgccagaggattatcctgatcagttcgatgatgtcatggattttattcaagccaccattaaaagactgaaaaggtcaccagataaacaaatggcagtgcttcctagaagagagcggaatcggcaggctgcagctgccaacccagagaattccagaggaaaaggtcggagaggccagaggggcaaaaaccggggttgtgtcttaactgcaatacatttaaatgtcactgacttgggtctgggctatgaaaccaaggaggaactgatttttaggtactgcagcggctcttgcgatgcagctgagacaacgtacgacaaaatattgaaaaacttatccagaaatagaaggctggtgagtgacaaagtagggcaggcatgttgcagacccatcgcctttgatgatgacctgtcgtttttagatgataacctggtttaccatattctaagaaagcattccgctaaaaggtgtggatgtatctgactccggctccagagactgctgtgtattgcattcctgctacagtgcaaagaaagggaccaaggttcccaggaaatgtttgcccagaatggaagatgaggaccaaggaggcggaggaggaggaagaagaagaggaggaggaggaggaggaggaggaggaggaggaaggcagccatcatgggagcctggtagagggagatccagctacagacaactggacaggagagagagaaaacagccctctggattctccaggatggcagccgatgtcactagaagctcagggctgatgttcctggttggctattgccaccatttcagctgatacagtccaccatcactgattaccggcgcggttgcggtggatgcacttgaaccaaaccagtgtatctcctgtgatttgttttcatgtgtccgaagacaccagggaaacagagatcctggtgttgttccttgttattacgttttactgctgaaagtaagaggtttatttttctgtcactcagtggagacataccctggaaaggagaggggaaaaaaaaagcaaagatacaagagataatcacctttgcatttgaaagttgaggcccgaggtttactacaaccagcatttttgccaacggttggtgattgatttccatcacggtgtgtggggtgggaagaagttggctaggaaccaaaaaggctgtgctcatgattaaacacaaacctgaaggtatttcctttatgtccttggaaacaggaaacgagttgtggttttcgccagcattcttgtaggagagaatcggggaaggccccgaactgcccccgggcagggagagcccctcaggcctgttggtttacagagagacagatgttacataaccagctccgttgatgcgtggtcaccagtgaccagagaagctactcgatgcaatgcatctgtttcagatacagaaatatagagaagatatttattgaaatttaagttattgttatttattaccgttcactaatgaatttctcttttttcccttatttattaaagtttcttttcaaaggtgccaaagtatatgtgctcgcaaaatgcaaagaaaggtgacaaaaggaaatttgaattgggaacaagggtccatgcttttcaaagtattaaaaagttttttgccaggcaaaaatcacttactttacctttttaagaaaatttgtcattaattttccccagatttcagcatttttcccaatttttatttgtggagcatctcaggcaagccccctttcctggagcagcgtgcagagaccactggcacttgactttatttcttccttgctccattgctgaacagaaatgtcgtgggctccacttcctgttgtctttaagctcttagtcccctccacgtatacctatctgtactatgcataaccatatgtagaaaaggttcagttccttttagtaggtagtcctggatttaatgctgacctaaaagtaatgtcgacaatgctgtcaggtagctgccgttctaccgactccctccatccctgcccacccactgccctcccgagaatatgctggctgcccagtgcagcccgggagacacaggggccttccagaggtagggtctaccaggtcctgtacaacccctgggctgtcaccgggggtcaacagctgctgctcctatatacccaaacacctgacagctccctggggagcagatggctgagaagggtgctgaggaagccatattgggaccagccacagccacacacatggagcctcatacttaggagcgtgctgcctttaaatgaaggtggtcggggccagtgcagcggctcacacccataatcccaacactttggaaagccaaggtgggaggatctcttgaacccaggagtttgagaccagcttgggcaacatagggagaccctgtctctacagaaactttaaaaattaggcaggcatgatggtgcacacctgtggtcccagctactcaagaggctgaaggaggatcacttgagtccagaaggtcgaggctgcagtgagctgtgatcatgccactgcactccagcctaagtgacagtgcggtaccctgtctcaaaaaaaaaaaaaaaaaaaaaaagaggttggagcaggaggaagcataggggcgggaacagccacctcctccatgccctagattgtgaatttatcgggcagccaacacatgtatgacacactaggccctgtattacagcttgttacgcatttcataaaagggattttcattaaggagataatctattactacctaccttagtggctactagtataaaactatgacagatttagcaattaaatgaaatactggcctccatcaaataatcatagtaacaagaagcagcagttaccagacatctgatccccttcccccaaaatacccaaattcttcatggttctgcccttctctgtcctttctgctccccttgctcgcctgggaaatggaggaaaggccttccctctcacactgtcttgggatcttgctgagaattcagactgctcgaaacagtgacaaaccccagccatccagtcattcgtggagcacaatttggatgtggccccaggggcatctgtcccattcagagaaccttggcagtgcgatggccactgttcccaggcttcaacctcagtgaccccccccaacaactccccatggagagtccctgcccaaaaaagctgtaggatccaaggggtgtcaatagctcgttcccggcatcacctacacaccacaagcaggttttaatggaagcaagttgctccaccaaatccacaaaagggtaaagtttgtgatttttctttatcattgcgatcaccatctgataccgtaaggagtgcacttgtttggaagttctgacttctctgatctgtcttggtcgtttgtgttataaaaccaaagttctctacagactttatttttgtacaatatcattttgtaactttttacaaataaaaactcatttctattgc

SEQ ID NO: 3 - protein, 15 aa, Homo sapiens
ETTYDKILKNLSRNR